European Patent Application EP 4 446 420 A1, published October 16, 2024. Title: L-lactic acid assimilating organisms and method for recycling resources using them. Applicant: NATIONAL UNIVERSITY CORPORATION KOBE UNIVERSITY. Application JP. The sequence listing filed with the application follows.

SEQUENCE LISTING (4 sequences)

SEQ ID NO: 1 - protein, 396 aa, Escherichia coli [sequence omitted]

SEQ ID NO: 2 - protein, 551 aa, Escherichia coli
MNLWQQNYDPAGNIWLSSLIASLPILFFFFALIKLKLKGYVAASWTVAIALAVALLFYKMPVANALASVVYGFFYGLWPIAWIIIAAVFVYKISVKTGQFDIIRSSILSITPDQRLQMLIVGFCFGAFLEGAAGFGAPVAITAALLVGLGFKPLYAAGLCLIVNTAPVAFGAMGIPILVAGQVTGIDSFEIGQMVGRQLPFMTIIVLFWIMAIMDGWRGIKETWPAVVVAGGSFAIAQYLSSNFIGPELPDIISSLVSLLCLTLFLKRWQPVRVFRFGDLGASQVDMTLAHTGYTAGQVLRAWTPFLFLTATVTLWSIPPFKALFASGGALYEWVINIPVPYLDKLVARMPPVVSEATAYAAVFKFDWFSATGTAILFAALLSIVWLKMKPSDAISTFGSTLKELALPIYSIGMVLAFAFISNYSGLSSTLALALAHTGHAFTFFSPFLGWLGVFLTGSDTSSNALFAALQATAAQQIGVSDLLLVAANTTGGVTGKMISPQSIAIACAAVGLVGKESDLFRFTVKHSLIFTCIVGVITTLQAYVLTWMIP

SEQ ID NO: 3 - DNA, 1191 bp, synthetic construct
  misc_feature 1..1191: note = E. coli lldD (codon optimized for Synechococcus elongatus)
  source 1..1191: mol_type = other DNA
atgatcatcagtgctgcctctgactatcgagcagctgctcagcgaattctacctcccttcctgttccactacatggatggtggtgcctactcggagtacaccctccgccgtaatgtcgaggatctgagtgaagtggcgctgcggcagcggattctgaagaacatgagcgacctctccttggaaaccaccctgttcaacgaaaaactctcgatgccggttgcgctagcgccagtaggtctctgtggcatgtacgcccgtcgcggtgaggtgcaagccgccaaagccgctgatgcccatggaattccatttactttatcgacggtgtcggtctgcccgattgaagaagttgctccggcgatcaagcgaccaatgtggtttcaactctacgtcctgcgcgatcgcggcttcatgcggaatgcccttgagcgggctaaagcggctggctgcagcacgctggtcttcacggtcgatatgcctactcccggcgctcgctatcgcgatgcccactccgggatgtccggccccaacgcagcgatgcgccgctatctccaggcagtcacccatccccagtgggcttgggatgttggcctcaatggacgtccccacgatctaggcaatatttcagcttatctgggtaagcccacgggtctggaggactacatcgggtggctgggtaacaactttgatcccagcatcagctggaaggatttagagtggattcgtgacttttgggacggtccgatggtgatcaaaggcattctcgatccggaagacgcgcgtgacgcagttcgctttggcgccgatggcatcgtggtcagcaatcatggcggtcgccaactggatggcgtgctgtcatctgctcgagcattgcctgctatcgctgatgctgtcaaaggcgatatcgcgatcttggcggacagtggaattcgcaatgggcttgatgtggttcggatgattgccttgggagcagacacagtgctcttggggcgcgcctttctctatgcccttgcgactgccgggcaagcgggcgttgccaatttgctcaacctgattgagaaagaaatgaaggtcgccatgaccttgacaggtgcgaaaagcatttctgaaatcacccaagatagtttggtacaggggctgggcaaggaactgcctgcggccttagcaccgatggccaagggcaacgctgcataa

SEQ ID NO: 4 - DNA, 1656 bp, synthetic construct
  misc_feature 1..1656: note = E. coli lldP (codon optimized Synechococcus elongatus)
  source 1..1656: mol_type = other DNA
atgaatctgtggcagcaaaactacgacccagcaggcaacatctggctgtcatcgcttattgcgtccttgccgattctgttcttcttctttgcattgatcaaactgaagctgaaaggctacgtcgcggcgagttggacggtggctattgctctggcagtggcgctgctcttctacaaaatgccggtcgccaatgccttagcgtctgttgtctatggctttttttacggcctttggccaattgcctggattatcattgcagcggtttttgtctacaagatttcggtcaaaaccgggcagtttgatatcattcgatcgtcgatattgagtatcaccccagatcagcgtctccaaatgctgattgtgggcttctgctttggggctttcctcgaaggggcagcagggtttggagcacccgtggcgattactgctgcgttgctggtcgggctgggttttaagcctctctatgcagccggactctgcttgatcgtcaatactgcccccgttgcctttggtgcgatgggcattcccatcttggtcgctggtcaagtcacgggaatcgacagttttgagattggtcagatggtggggcggcaactccctttcatgacgatcatcgttctgttttggatcatggcgattatggatggctggcgaggtatcaaggaaacctggccggcggtagtggtggccggcgggagcttcgcgatcgcccagtatctcagcagcaactttatcggtcctgaactgcccgatattatttctagtctggttagcttgctttgtctgactctgttcctcaaacgctggcaaccggttcgtgtcttccgctttggcgatttgggagccagccaggttgatatgaccctagcccatacgggttataccgcgggccaagtgctgcgcgcttggacccccttcctctttctcacggccaccgtaacgctctggagcataccgcctttcaaagcactgtttgcctcgggaggtgccctctacgagtgggtgattaatattccggtgccctatcttgacaagttggtggcacggatgcccccagttgtcagcgaagccacagcctacgccgcagtgttcaagtttgactggttttcagccacgggaacagccattctttttgctgctcttctcagtattgtttggctcaagatgaaaccgagcgatgcgatcagtaccttcggctctacgctaaaagagttagctctaccgatctacagcattgggatggtcctagcatttgcctttatcagcaattattcaggcctgtcttcaacactggccttggctttggcccatacaggccacgcgttcacctttttctcgccctttttaggttggctgggcgtctttctgaccggttccgacaccagctccaacgctttgttcgcggcactgcaggctactgcagcccaacagattggtgtcagtgatttgctgttggtggctgctaacacgaccggcggcgtgactggcaagatgatctccccccagtcgatcgcaatcgcttgtgctgctgtgggcttagttggcaaagaaagcgatttgtttcgcttcacggtcaagcactccctgatcttcacctgcatcgttggtgtgatcaccacactacaagcctatgtgttgacttggatgattccttaa